European Patent Specification EP 3 512 858 B1, published November 8, 2023. Title: FUSED BICYCLIC INHIBITORS OF MENIN-MLL INTERACTION. Applicant: Janssen Pharmaceutica NV. The sequence listing filed with the application follows.

SEQUENCE LISTING (1 sequence)

SEQ ID NO: 1 - protein, 616 aa, Artificial Sequence
  MENIN protein sequence with His tag
MGLKAAQKTLFPLRSIDDVVRLFAAELGREEPDLVLLSLVLGFVEHFLAVNRVIPTNVPELTFQPSPAPDPPGGLTYFPVADLSIIAALYARFTAQIRGAVDLSLYPREGGVSSRELVKKVSDVIWNSLSRSYFKDRAHIQSLFSFITGTKLDSSGVAFAVVGACQALGLRDVHLALSEDHAWVVFGPNGEQTAEVTWHGKGNEDRRGQTVNAGVAERSWLYLKGSYMRCDRKMEVAFMVCAINPSIDLHTDSLELLQLQQKLLWLLYDLGHLERYPMALGNLADLEELEPTPGRPDPLTLYHKGIASAKTYYRDEHIYPYMYLAGYHCRNRNVREALQAWADTATVIQDYNYCREDEEIYKEFFEVANDVIPNLLKEAASLLEAGEERPGEQSQGTQSQGSALQDPECFAHLLRFYDGICKWEEGSPTPVLHVGWATFLVQSLGRFEGQVRQKVRIVSREAEAAEAEEPWGEEAREGRRRGPRRESKPEEPPPPKKPALDKGLGTGQGAVSGPPRKPPGTVAGTARGPEGGSTAQVPAPAASPPPEGPVLTFQSEKMKGMKELLVATKINSSAIKLQLTAQSQVQMKKQKVSTPSDYTLSFLKRQRKGLHHHHHH